European Patent Application EP 4 169 945 A1, published April 26, 2023. Title: TRANSFORMING GROWTH FACTOR-BETA-RESPONSIVE POLYPEPTIDES AND THEIR METHODS FOR USE. Applicant: The Regents of the University of California. Application EP, filed October 28, 2016. The sequence listing filed with the application follows.

SEQUENCE LISTING (101 sequences)

SEQ ID NO: 1 - protein, 124 aa, synthetic construct
EVQLVESGGGLVQPGGSLRLSCAASGYAFTNYLIEWVRQAPGKGLEWVGVINPGSGGSNYNEKFKGRATISADNSKNTLYLQMNSLRAEDTAVYYCARSGGFYFDYWGQGTLVTVSSASTKGPS

SEQ ID NO: 2 - protein, 116 aa, synthetic construct
DIQMTQSPSSLSASVGDRVTITCRASQSVLYSSNQKNYLAWYQQKPGKAPKLLIYWASTRESGVPSRFSGSGSGTDFTLTISSLQPEDFATYYCHQYLSSDTFGQGTKVEIKRTVA

SEQ ID NO: 3 - protein, 120 aa, synthetic construct
QVQLVQSGAEVKKPGSSVKVSCKASGYTFSSNVISWVRQAPGQGLEWMGGVIPIVDIANYAQRFKGRVTITADESTSTTYMELSSLRSEDTAVYYCALPRAFVLDAMDYWGQGTLVTVSS

SEQ ID NO: 4 - protein, 108 aa, synthetic construct
ETVLTQSPGTLSLSPGERATLSCRASQSLGSSYLAWYQQKPGQAPRLLIYGASSRAPGIPDRFSGSGSGTDFTLTISRLEPEDFAVYYCQQYADSPITFGQGTRLEIK

SEQ ID NO: 5 - protein, 10 aa, synthetic construct
GYAFTNYLIE

SEQ ID NO: 6 - protein, 17 aa, synthetic construct
VINPGSGGSNYNEKFKG

SEQ ID NO: 7 - protein, 8 aa, synthetic construct
SGGFYFDY

SEQ ID NO: 8 - protein, 17 aa, synthetic construct
RASQSVLYSSNQKNYLA

SEQ ID NO: 9 - protein, 7 aa, synthetic construct
WASTRES

SEQ ID NO: 10 - protein, 8 aa, synthetic construct
HQYLSSDT

SEQ ID NO: 11 - protein, 5 aa, synthetic construct
SNVIS

SEQ ID NO: 12 - protein, 17 aa, synthetic construct
GVIPIVDIANYAQRFKG

SEQ ID NO: 13 - protein, 11 aa, synthetic construct
PRAFVLDAMDY

SEQ ID NO: 14 - protein, 12 aa, synthetic construct
RASQSLGSSYLA

SEQ ID NO: 15 - protein, 7 aa, synthetic construct
GASSRAP

SEQ ID NO: 16 - protein, 9 aa, synthetic construct
QQYADSPIT

SEQ ID NO: 17 - protein, 8 aa, synthetic construct
DYKDDDDK

SEQ ID NO: 18 - protein, 20 aa, synthetic construct
METDTLLLWVLLLWVPGSTG

SEQ ID NO: 19 - protein, 123 aa, synthetic construct
EVQLVESGGGVVQPGRSLRLSCAASGFTFSSYGMHWVRQAPGKELEWVAVISYDGSIKYYADSVKGRFTISRDNSKNTLYLQMNSLRAEDTAVYYCARTGEYSGYDTDPQYSWGQGTTVTVSS

SEQ ID NO: 20 - protein, 107 aa, synthetic construct
EIVLTQSPSSLSASVGDRVTITCRSSQGIGDDLGWYQQKPGKAPILLIYGTSTLQSGVPSRFSGSGSGTDFTLTINSLQPEDFATYYCLQDSNYPLTFGGGTRLEIK

SEQ ID NO: 21 - protein, 5 aa, synthetic construct
SYGMH

SEQ ID NO: 22 - protein, 17 aa, synthetic construct
VISYDGSIKYYADSVKG

SEQ ID NO: 23 - protein, 14 aa, synthetic construct
TGEYSGYDTDPQYS

SEQ ID NO: 24 - protein, 11 aa, synthetic construct
RSSQGIGDDLG

SEQ ID NO: 25 - protein, 7 aa, synthetic construct
GTSTLQS

SEQ ID NO: 26 - protein, 9 aa, synthetic construct
LQDSNYPLT

SEQ ID NO: 27 - protein, 5 aa, synthetic construct
DKTHT

SEQ ID NO: 28 - protein, 4 aa, synthetic construct
CPPC

SEQ ID NO: 29 - protein, 15 aa, synthetic construct
CPEPKSCDTPPPCPR

SEQ ID NO: 30 - protein, 12 aa, synthetic construct
ELKTPLGDTTHT

SEQ ID NO: 31 - protein, 10 aa, synthetic construct
KSCDKTHTCP

SEQ ID NO: 32 - protein, 7 aa, synthetic construct
KCCVDCP

SEQ ID NO: 33 - protein, 7 aa, synthetic construct
KYGPPCP

SEQ ID NO: 34 - protein, 15 aa, synthetic construct
EPKSCDKTHTCPPCP

SEQ ID NO: 35 - protein, 12 aa, synthetic construct
ERKCCVECPPCP

SEQ ID NO: 36 - protein, 17 aa, synthetic construct
ELKTPLGDTTHTCPRCP

SEQ ID NO: 37 - protein, 12 aa, synthetic construct
SPNMVPHAHHAQ

SEQ ID NO: 38 - protein, 15 aa, synthetic construct
EPKSCDKTYTCPPCP

SEQ ID NO: 39 - protein, 45 aa, synthetic construct
TTTPAPRPPTPAPTIASQPLSLRPEACRPAAGGAVHTRGLDFACD

SEQ ID NO: 40 - protein, 5 aa, synthetic construct
  REGION >5: note = amino acids 1-5 repeated more than once
GSGGS

SEQ ID NO: 41 - protein, 4 aa, synthetic construct
  REGION >4: note = amino acids 1-4 repeated more than once
GGGS

SEQ ID NO: 42 - protein, 4 aa, synthetic construct
GGSG

SEQ ID NO: 43 - protein, 5 aa, synthetic construct
GGSGG

SEQ ID NO: 44 - protein, 5 aa, synthetic construct
GSGSG

SEQ ID NO: 45 - protein, 5 aa, synthetic construct
GSGGG

SEQ ID NO: 46 - protein, 5 aa, synthetic construct
GGGSG

SEQ ID NO: 47 - protein, 5 aa, synthetic construct
GSSSG

SEQ ID NO: 48 - protein, 24 aa, synthetic construct
IYIWAPLAGTCGVLLLSLVITLYC

SEQ ID NO: 49 - protein, 23 aa, synthetic construct
LGLLVAGVLVLLVSLGVAIHLCC

SEQ ID NO: 50 - protein, 25 aa, synthetic construct
ALIVLGGVAGLLLFIGLGIFFCVRC

SEQ ID NO: 51 - protein, 23 aa, synthetic construct
LCYLLDGILFIYGVILTALFLRV

SEQ ID NO: 52 - protein, 26 aa, synthetic construct
WVLVVVGGVLACYSLLVTVAFIIFWV

SEQ ID NO: 53 - protein, 26 aa, synthetic construct
VAAILGLGLVLGLLGPLAILLALYLL

SEQ ID NO: 54 - protein, 24 aa, synthetic construct
ALPAALAVISFLLGLGLGVACVLA

SEQ ID NO: 55 - protein, 42 aa, synthetic construct
KRGRKKLLYIFKQPFMRPVQTTQEEDGCSCRFPEEEEGGCEL

SEQ ID NO: 56 - protein, 44 aa, synthetic construct
FWVRSKRSRLLHSDYMNMTPRRPGPTRKHYQPYAPPRDFAAYRS

SEQ ID NO: 57 - protein, 35 aa, synthetic construct
TKKKYSSSVHDPNGEYMFMRAVNTAKKSRLTDVTL

SEQ ID NO: 58 - protein, 37 aa, synthetic construct
RRDQRLPPDAHKPPGGGSFRTPIQEEQADAHSTLAKI

SEQ ID NO: 59 - protein, 114 aa, synthetic construct
  REGION 1..114: note = Synthetic Peptide
CCLRRHQGKQNELSDTAGREINLVDAHLKSEQTEASTRQNSQVLLSETGIYDNDPDLCFRMQEGSEVYSNPCLEENKPGIVYASLNHSVIGPNSRLARNVKEAPTEYASICVRS

SEQ ID NO: 60 - protein, 49 aa, synthetic construct
HQRRKYRSNKGESPVEPAEPCRYSCPREEEGSTIPIQEDYRKPEPACSP

SEQ ID NO: 61 - protein, 187 aa, synthetic construct
RRACRKRIRQKLHLCYPVQTSQPKLELVDSRPRRSSTQLRSGASVTEPVAEERGLMSQPLMETCHSVGAAYLESLPLQDASPAGGPSSPRDLPEPRVSTEHTNNKIEKIYIMKADTVIVGTVKAELPEGRGLAGPAEPELEEELEADHTPHYPEQETEPPLGSCSDVMLSVEEEGKEDPLPTAASGK

SEQ ID NO: 62 - protein, 54 aa, synthetic construct
HIWQLRSQCMWPRETQLLLEVPPSTEDARSCQFPEEERGERSAEEKGRLGDLWV

SEQ ID NO: 63 - protein, 60 aa, synthetic construct
CVKRRKPRGDVVKVIVSVQRKRQEAEGEATVIEALQAPPDVTTVAVEETIPSFTGRSPNH

SEQ ID NO: 64 - skipped

SEQ ID NO: 65 - protein, 16 aa, synthetic construct
  VARIANT 2..3: note = X is A, C, D, E, F, G, H, I, K, L, M, N, P, Q, R, S, T, V, W or Y
  VARIANT 5..12: note = X is A, C, D, E, F, G, H, I, K, L, M, N, P, Q, R, S, T, V, W or Y, or absent
  VARIANT 14..15: note = X is A, C, D, E, F, G, H, I, K, L, M, N, P, Q, R, S, T, V, W or Y
YXXJXXXXXXXXYXXJ

SEQ ID NO: 66 - protein, 113 aa, synthetic construct
MGGLEPCSRLLLLPLLLAVSGLRPVQAQAQSDCSCSTVSPGVLAGIVMGDLVLTVLIALAVYFLGRLVPRGRGAAEAATRKORITETESPYOELOGORSDVYSDLNTQRPYYK

SEQ ID NO: 67 - protein, 112 aa, synthetic construct
MGGLEPCSRLLLLPLLLAVSGLRPVQAQAQSDCSCSTVSPGVLAGIVMGDLVLTVLIALAVYFLGRLVPRGRGAAEATRKORITETESPYOELOGORSDVYSDLNTQRPYYK

SEQ ID NO: 68 - protein, 102 aa, synthetic construct
MGGLEPCSRLLLLPLLLAVSDCSCSTVSPGVLAGIVMGDLVLTVLIALAVYFLGRLVPRGRGAAEAATRKORITETESPYOELOGORSDVYSDLNTQRPYYK

SEQ ID NO: 69 - protein, 101 aa, synthetic construct
MGGLEPCSRLLLLPLLLAVSDCSCSTVSPGVLAGIVMGDLVLTVLIALAVYFLGRLVPRGRGAAEATRKORITETESPYOELOGORSDVYSDLNTQRPYYK

SEQ ID NO: 70 - protein, 21 aa, synthetic construct
ESPYOELOGORSDVYSDLNTO

SEQ ID NO: 71 - protein, 86 aa, synthetic construct
MIPAVVLLLLLLVEQAAALGEPQLCYILDAILFLYGIVLTLLYCRLKIQVRKAAITSYEKSDGVYTGLSTRNQETYETLKHEKPPQ

SEQ ID NO: 72 - protein, 21 aa, synthetic construct
DGVYTGLSTRNOETYETLKHE

SEQ ID NO: 73 - protein, 171 aa, synthetic construct
MEHSTFLSGLVLATLLSQVSPFKIPIEELEDRVFVNCNTSITWVEGTVGTLLSDITRLDLGKRILDPRGIYRCNGTDIYKDKESTVQVHYRMCQSCVELDPATVAGIIVTDVIATLLLALGVFCFAGHETGRLSGAADTOALLRNDOVYOPLRDRDDAOYSHLGGNWARNK

SEQ ID NO: 74 - protein, 127 aa, synthetic construct
MEHSTFLSGLVLATLLSQVSPFKIPIEELEDRVFVNCNTSITWVEGTVGTLLSDITRLDLGKRILDPRGIYRCNGTDIYKDKESTVOVHYRTADTOALLRNDOVYOPLRDRDDAQYSHLGGNWARNK

SEQ ID NO: 75 - protein, 21 aa, synthetic construct
DOVYOPLRDRDDAOYSHLGGN

SEQ ID NO: 76 - protein, 207 aa, synthetic construct
MQSGTHWRVLGLCLLSVGVWGQDGNEEMGGITQTPYKVSISGTTVILTCPQYPGSEILWQHNDKNIGGDEDDKNIGSDEDHLSLKEFSELEQSGYYVCYPRGSKPEDANFYLYLRARVCENCMEMDVMSVATIVIVDICITGGLLLLVYYWSKNRKAKAKPVTRGAGAGGRQRGQNKERPPPVPNPDYEPIRKGQRDLYSGLNQRRI

SEQ ID NO: 77 - protein, 21 aa, synthetic construct
NPDYEPIRKGQRDLYSGLNQR

SEQ ID NO: 78 - protein, 182 aa, synthetic construct
MEQGKGLAVLILAIILLQGTLAQSIKGNHLVKVYDYQEDGSVLLTCDAEAKNITWFKDGKMIGFLTEDKKKWNLGSNAKDPRGMYQCKGSQNKSKPLQVYYRMCQNCIELNAATISGFLFAEIVSIFVLAVGVYFIAGODGVROSRASDKOTLLPNDOLYOPLKDREDDQYSHLQGNQLRRN

SEQ ID NO: 79 - protein, 21 aa, synthetic construct
DOLYOPLKDREDDOYSHLOGN

SEQ ID NO: 80 - protein, 163 aa, synthetic construct
MKWKALFTAAILQAQLPITEAQSFGLLDPKLCYLLDGILFIYGVILTALFLRVKFSRSADAPAYQQGQNQLYNELNLGRREEYDVLDKRRGRDPEMGGKPRRKNPQEGLYNELOKDKMAEAYSEIGMKGERRRGKGHDGLYOGLSTATKDTYDALHMQALPPR

SEQ ID NO: 81 - protein, 164 aa, synthetic construct
MKWKALFTAAILQAQLPITEAQSFGLLDPKLCYLLDGILFIYGVILTALFLRVKFSRSADAPAYQQGQNQLYNELNLGRREEYDVLDKRRGRDPEMGGKPQRRKNPQEGLYNELOKDKMAEAYSEIGMKGERRRGKGHDGLYOGLSTATKDTYDALHMQALPPR

SEQ ID NO: 82 - protein, 112 aa, synthetic construct
RVKFSRSADAPAYOQGONOLYNELNLGRREEYDVLDKRRGRDPEMGGKPRRKNPOEGLYNELOKDKMAEAYSEIGMKGERRRGKGHDGLYOGLSTATKDTYDALHMQALPPR

SEQ ID NO: 83 - protein, 21 aa, synthetic construct
NOLYNELNLGRREEYDVLDKR

SEQ ID NO: 84 - protein, 22 aa, synthetic construct
EGLYNELQKDKMAEAYSEIGMK

SEQ ID NO: 85 - protein, 21 aa, synthetic construct
DGLYOGLSTATKDTYDALHMO

SEQ ID NO: 86 - protein, 226 aa, synthetic construct
MPGGPGVLQALPATIFLLFLLSAVYLGPGCQALWMHKVPASLMVSLGEDAHFQCPHNSSNNANVTWWRVLHGNYTWPPEFLGPGEDPNGTLIIQNVNKSHGGIYVCRVQEGNESYQQSCGTYLRVRQPPPRPFLDMGEGTKNRIITAEGIILLFCAVVPGTLLLFRKRWONEKLGLDAGDEYEDENLYEGLNLDDCSMYEDISRGLOGTYQDVGSLNIGDVQLEKP

SEQ ID NO: 87 - protein, 188 aa, synthetic construct
MPGGPGVLQALPATIFLLFLLSAVYLGPGCQALWMHKVPASLMVSLGEDAHFQCPHNSSNNANVTWWRVLHGNYTWPPEFLGPGEDPNEPPPRPFLDMGEGTKNRIITAEGIILLFCAVVPGTLLLFRKRWQNEKLGLDAGDEYEDENLYEGLNLDDCSMYEDISRGLQGTYQDVGSLNIGDVQLEKP

SEQ ID NO: 88 - protein, 21 aa, synthetic construct
ENLYEGLNLDDCSMYEDISRG

SEQ ID NO: 89 - protein, 20 aa, synthetic construct
RPRRSPAQDGKVYINMPGRG

SEQ ID NO: 90 - protein, 20 aa, synthetic construct
RPRRSPAQDGKVYINMPGRG

SEQ ID NO: 91 - protein, 68 aa, synthetic construct
FWVLVVVGGVLACYSLLVTVAFIIFWVRSKRSRLLHSDYMNMTPRRPGPTRKHYQPYAPPRDFAAYRS

SEQ ID NO: 92 - protein, 68 aa, synthetic construct; identical to SEQ ID NO: 91

SEQ ID NO: 93 - protein, 619 aa, synthetic construct
MPDPAAHLPFFYGSISRAEAEEHLKLAGMADGLFLLRQCLRSLGGYVLSLVHDVRFHHFPIERQLNGTYAIAGGKAHCGPAELCEFYSRDPDGLPCNLRKPCNRPSGLEPQPGVFDCLRDAMVRDYVRQTWKLEGEALEQAIISQAPQVEKLIATTAHERMPWYHSSLTREEAERKLYSGAQTDGKFLLRPRKEQGTYALSLIYGKTVYHYLISQDKAGKYCIPEGTKFDTLWQLVEYLKLKADGLIYCLKEACPNSSASNASGAAAPTLPAHPSTLTHPQRRIDTLNSDGYTPEPARITSPDKPRPMPMDTSVYESPYSDPEELKDKKLFLKRDNLLIADIELGCGNFGSVRQGVYRMRKKQIDVAIKVLKQGTEKADTEEMMREAQIMHQLDNPYIVRLIGVCQAEALMLVMEMAGGGPLHKFLVGKREEIPVSNVAELLHQVSMGMKYLEEKNFVHRDLAARNVLLVNRHYAKISDFGLSKALGADDSYYTARSAGKWPLKWYAPECINFRKFSSRSDVWSYGVTMWEALSYGQKPYKKMKGPEVMAFIEQGKRMECPPECPPELYALMSDCWIYKWEDRPDFLTVEQRMRACYYSLASKVEGPPGSTQKAEAACA

SEQ ID NO: 94 - protein, 9 aa, synthetic construct
YPYDVPDYA

SEQ ID NO: 95 - protein, 10 aa, synthetic construct
EQKLISEEDL

SEQ ID NO: 96 - protein, 290 aa, synthetic construct
METDTLLLWVLLLWVPGSTGAGGSDYKDDDDKGGSEVQLVESGGGLVQPGGSLRLSCAASGYAFTNYLIEWVRQAPGKGLEWVGVINPGSGGSNYNEKFKGRATISADNSKNTLYLQMNSLRAEDTAVYYCARSGGFYFDYWGQGTLVTVSSASTKGPSGGGGSGGGGSGGGGSDIQMTQSPSSLSASVGDRVTITCRASQSVLYSSNQKNYLAWYQQKPGKAPKLLIYWASTRESGVPSRFSGSGSGTDFTLTISSLQPEDFATYYCHQYLSSDTFGQGTKVEIKRTVA

SEQ ID NO: 97 - protein, 278 aa, synthetic construct
METDTLLLWVLLLWVPGSTGAGGSDYKDDDDKGGSQVQLVQSGAEVKKPGSSVKVSCKASGYTFSSNVISWVRQAPGQGLEWMGGVIPIVDIANYAQRFKGRVTITADESTSTTYMELSSLRSEDTAVYYCALPRAFVLDAMDYWGQGTLVTVSSGGGGSGGGGSGGGGSETVLTQSPGTLSLSPGERATLSCRASQSLGSSYLAWYQQKPGQAPRLLIYGASSRAPGIPDRFSGSGSGTDFTLTISRLEPEDFAVYYCQQYADSPITFGQGTRLEIK

SEQ ID NO: 98 - protein, 12 aa, synthetic construct
ESKYGPPCPPCP

SEQ ID NO: 99 - protein, 12 aa, synthetic construct
ESKYGPPCPSCP

SEQ ID NO: 100 - protein, 246 aa, synthetic construct
DIVLTQSPAILSASPGEKVTMTCRASSSVNYMDWYQKKPGSSPKPWIYATSNLASGVPARFSGSGSGTSYSLTISRVEAEDAATYYCQQWSFNPPTFGGGTKLEIKGSTSGGGSGGGSGGGGSSEVQLQQSGAELVKPGASVKMSCKASGYTFTSYNMHVWKQTPGQGLEWIGAIYPGNGDTSYNQKFKGKATLTADKSSSTAYMQLSSLTSEDSADYYCARSNYYGSSYWFFDVWGAGTTVTVSS

SEQ ID NO: 101 - protein, 245 aa, synthetic construct
DIQMTQTTSSLSASLGDRVTISCRASQDISKYLNWYQQKPDGTVKLLIYHTSRLHSGVPSRFSGSGSGTDYSLTISNLEQEDIATYFCQQGNTLPYTFGGGTKLEITGSTSGSGKPGSGEGSTKGEVKLQESGPGLVAPSQSLSVTCTVSGVSLPDYGVSWIRQPPRKGLEWLGVIWGSETTYYNSALKSRLTIIKDNSKSQVFLKMNSLQTDDTAIYYCAKHYYYGGSYAMDYWGQGTSVTVSS